European Patent Application EP 4 462 114 A1, published November 13, 2024. Title: Methods for identifying sugar-bound amino acid site in protein, and kit. Applicant: FUJIFILM Corporation. The sequence listing filed with the application follows.

SEQUENCE LISTING (3 sequences)

SEQ ID NO: 1 - protein, 14 aa, Adeno-associated virus
FSVAGPSNMAVQGR

SEQ ID NO: 2 - protein, 14 aa, Adeno-associated virus
  SITE 7: note = misc_feature - Xaa represents GlcNAc-bound Serine.
FSVAGPXNMAVQGR

SEQ ID NO: 3 - protein, 26 aa, Adeno-associated virus
VSTTVTQNNNSEFAWPGASSWALNGR